European Patent Specification EP 3 193 584 B1, published September 4, 2024. Title: Stay green cucumber plant. Applicant: Enza Zaden Beheer B.V. The sequence listing filed with the application follows.

SEQUENCE LISTING (4 sequences)

SEQ ID NO: 1 - DNA, 2501 bp, Cucumis sativus
  source 1..2501: /mol_type="unassigned DNA" /organism="Cucumis sativus"
tgcttgtatttttgggtcaaataacagattaatgtaaataaaattcgatatggaagtttgaaagcatttagatagaatagcatgtagtctaaaaatgtatttagtggccggtagagtatacaagtatttgtagtgggtagcatccaaagtcaaaaacagagacggtgtcgtattattgatcaaccacgtaaaatcccccaaaggaaaaataatggttgcttattacaaccaaacctaaacgaagtctactacttgaagcaacagcgaagaaaaagcaattcctttcctacacgcttctaattcccaaaaattctggacttcactactcatcagattatacacagcatttcctttttcattcttccccttttctcttttttctttttttcttttgtttcccataagcctcatattttgttcctccctaagtttcctctgtttttgatcctttaaaccgatcacaaaccctcccaaatttctggagctaatttgttggacaagatgagggttttgactggtaattcttctcctcttcttgttccttcttcaaacccttatcacgattcttcttctctcttcccctgtaaacgcaaatccaagaagaagaaccatggaatggttcctgtaagtttctttctttctttctttctttttttgggttttgttttggttttgattttgattttgactctgattttaattttatagatggcgagattgtttgggccagccatatttgaagcttcgaagctaaaggttctgtttttaggggtggatgagaagaaacatccaggcaaatttccaaggacttatacgctcacacatagtgatattacttctaaacttactcttgccatttctcaatccattaacaattctcaggtaactcttcttcttcttcttctttttagtttaatgaaaactccttttctagtttgtcaaatatttgaaaattgatagttttgttttagattataattatgtgaaacgtgttttttattcttgaataatgcttctcatatcagatacttattgatttttttcttcttttccttttttatttagcttgaagacacttcttcaatattttttaaaataaaatttaccaatatttagaaaaaaaagaaaacaaagctatagttttgaaaacttaaaaatagtttacaaaactatatcttctcggtattttgaatctgaattctattttaaaatttggttagaaattcaagtttttttaagaaaagtgaccgaatagagttttgaagtcccaacaatccaactatatgggaactttattttctggaatgggtgttaaatacaataaaaatgtaagtattgatgatgatggatgaatatattattacgcagttacaaggatggtataattggcttcaaagggatgaagtggtaggagaatggaagaaagttaagggaaaaatgtctcttcatgttcattgtcatatcagtggtggccattttcttctagatctttgtgctaatctcagatacttcatctttcgcaaagaactccctgtggtaatttctctttctcttcatctattatttactataagatgcacaaaaactacaggataaagaatagactccaatcattgatctatgagaagttagatataaattttacactatcagcaaattacttgcatttggatcatttgatgtctgctatttttcatttacttgtccaataaaaaaattataatacataccccacttctgaataatttattatataattgacatttgattcacacgatataaaggtgttgaatgctttcgtccatggagatgtggatttattcaacaattaccctgaattacaagaggctatggtttgggtttatttccactccaaaattccagaattcaacaaggtagagtgttggggcccactgaaggatccagccccaccttcaactgggcttgatgggtccactcaaagccagcccatgtgggaattgggcttgctggagcggcccaaaccttgtcaagaagattgcacttgttgcttcccaaccatcccttccatttcatggtctcccaagaataatgagttggagagcacatagattcattttattgactgcccttaaaatgtaaatagttcatctttattgttactatataatgacaattgaatgttttcaactttctatttagtccttatatttcaattcgttaatctttgtagtatctaagatgttaaattatatatcgtggaaattttcttctttcaatagtgtttttgatgaaatataaggaaatttctcgttatgtttcgatgaaatcttttttctagttttaattatatcatgaatttgtaataaccgagctaagattgtagaaaaacaagttagacagttgtatgttgcagacttgtgaattcctgcatgctttggagggattggtaaaattcttttaaaaaagggaaagaaatgcttatatgcataaggaagaattgacacaatatgctaccagta

SEQ ID NO: 2 - protein, 256 aa, Cucumis sativus
MRVLTGNSSPLLVPSSNPYHDSSSLFPCKRKSKKKNHGMVPMARLFGPAIFEASKLKVLFLGVDEKKHPGKFPRTYTLTHSDITSKLTLAISQSINNSQLQGWYNWLQRDEVVGEWKKVKGKMSLHVHCHISGGHFLLDLCANLRYFIFRKELPVVLNAFVHGDVDLFNNYPELQEAMVWVYFHSKIPEFNKVECWGPLKDPAPPSTGLDGSTQSQPMWELGLLERPKPCQEDCTCCFPTIPSISWSPKNNELEST

SEQ ID NO: 3 - DNA, 2501 bp, Cucumis sativus
  source 1..2501: /mol_type="unassigned DNA" /organism="Cucumis sativus"
tgcttgtatttttgggtcaaataacagattaatgtaaataaaattcgatatggaagtttgaaagcatttagatagaatagcatgtagtctaaaaatgtatttagtggccggtagagtatacaagtatttgtagtgggtagcatccaaagtcaaaaacagagacggtgtcgtattattgatcaaccacgtaaaatcccccaaaggaaaaataatggttgcttattacaaccaaacctaaacgaagtctactacttgaagcaacagcgaagaaaaagcaattcctttcctacacgcttctaattcccaaaaattctggacttcactactcatcagattatacacagcatttcctttttcattcttccccttttctcttttttctttttttcttttgtttcccataagcctcatattttgttcctccctaagtttcctctgtttttgatcctttaaaccgatcacaaaccctcccaaatttctggagctaatttgttggacaagatgagggttttgactggtaattcttctcctcttcttgttccttcttcaaacccttatcacgattcttcttctctcttcccctgtaaacgcaaatccaagaagaagaaccatggaatggttcctgtaagtttctttctttctttctttctttttttgggttttgttttggttttgattttgattttgactctgattttaattttatagatggcgagattgtttgggccagccatatttgaagcttcgaagctaaaggttctgtttttaggggtggatgagaagaaacatccaggcaaatttccaaggacttatacgctcacacatagtgatattacttctaaacttactcttgccatttctcaatccattaacaattctcaggtaactcttcttcttcttcttctttttagtttaatgaaaactccttttctagtttgtcaaatatttgaaaattgatagttttgttttagattataattatgtgaaacgtgttttttattcttgaataatgcttctcatatcagatacttattgatttttttcttcttttccttttttatttagcttgaagacacttcttcaatattttttaaaataaaatttaccaatatttagaaaaaaaagaaaacaaagctatagttttgaaaacttaaaaatagtttacaaaactatatcttctcggtattttgaatctgaattctattttaaaatttggttagaaattcaagtttttttaagaaaagtgaccgaatagagttttgaagtcccaacaatccaactatatgggaactttattttctggaatgggtgttaaatacaataaaaatgtaagtattgatgatgatggatgaatatattattacgcagttacaaggatggtataattggcttcaaagggatgaagtggtaggagaatggaagaaagttaagggaaaaatgtctcttcatgttcattgtcatatcagtggtggccattttcttctagatctttgtgctaatctcagatacttcatctttcgcaaagaattccctgtggtaatttctctttctcttcatctattatttactataagatgcacaaaaactacaggataaagaatagactccaatcattgatctatgagaagttagatataaattttacactatcagcaaattacttgcatttggatcatttgatgtctgctatttttcatttacttgtccaataaaaaaattataatacataccccacttctgaataatttattatataattgacatttgattcacacgatataaaggtgttgaatgctttcgtccatggagatgtggatttattcaacaattaccctgaattacaagaggctatggtttgggtttatttccactccaaaattccagaattcaacaaggtagagtgttggggcccactgaaggatccagccccaccttcaactgggcttgatgggtccactcaaagccagcccatgtgggaattgggcttgctggagcggcccaaaccttgtcaagaagattgcacttgttgcttcccaaccatcccttccatttcatggtctcccaagaataatgagttggagagcacatagattcattttattgactgcccttaaaatgtaaatagttcatctttattgttactatataatgacaattgaatgttttcaactttctatttagtccttatatttcaattcgttaatctttgtagtatctaagatgttaaattatatatcgtggaaattttcttctttcaatagtgtttttgatgaaatataaggaaatttctcgttatgtttcgatgaaatcttttttctagttttaattatatcatgaatttgtaataaccgagctaagattgtagaaaaacaagttagacagttgtatgttgcagacttgtgaattcctgcatgctttggagggattggtaaaattcttttaaaaaagggaaagaaatgcttatatgcataaggaagaattgacacaatatgctaccagta

SEQ ID NO: 4 - protein, 256 aa, Cucumis sativus
MRVLTGNSSPLLVPSSNPYHDSSSLFPCKRKSKKKNHGMVPMARLFGPAIFEASKLKVLFLGVDEKKHPGKFPRTYTLTHSDITSKLTLAISQSINNSQLQGWYNWLQRDEVVGEWKKVKGKMSLHVHCHISGGHFLLDLCANLRYFIFRKEFPVVLNAFVHGDVDLFNNYPELQEAMVWVYFHSKIPEFNKVECWGPLKDPAPPSTGLDGSTQSQPMWELGLLERPKPCQEDCTCCFPTIPSISWSPKNNELEST